European Patent Specification EP 4 051 708 B1, published January 8, 2025. Title: TSLP BINDING MOLECULES AND USES THEREOF. Applicant: MEDIMMUNE LIMITED. The sequence listing filed with the application follows.

SEQUENCE LISTING (31 sequences)

SEQ ID NO: 1 - protein, 5 aa, Homo sapiens
  MISC_FEATURE: HCDR1 FAB1
TYGMH

SEQ ID NO: 2 - protein, 17 aa, Homo sapiens
  MISC_FEATURE: HCDR2 FAB1
VIWYDGSNKHYADSVKG

SEQ ID NO: 3 - protein, 13 aa, Homo sapiens
  MISC_FEATURE: HCDR3 FAB1
APQWELVHEAFDI

SEQ ID NO: 4 - protein, 122 aa, Homo sapiens
  MISC_FEATURE: HEAVY CHAIN VH FAB1
QMQLVESGGGVVQPGRSLRLSCAASGFTFRTYGMHWVRQAPGKGLEWVAVIWYDGSNKHYADSVKGRFTITRDNSKNTLNLQMNSLRAEDTAVYYCARAPQWELVHEAFDIWGQGTMVTVSS

SEQ ID NO: 5 - protein, 11 aa, Homo sapiens
  MISC_FEATURE: LCDR1 FAB1
GGNNLGSKSVH

SEQ ID NO: 6 - protein, 7 aa, Homo sapiens
  MISC_FEATURE: LCDR2 FAB1
DDSDRPS

SEQ ID NO: 7 - protein, 11 aa, Homo sapiens
  MISC_FEATURE: LCDR3 FAB1
QVWDSSSDHVV

SEQ ID NO: 8 - protein, 108 aa, Homo sapiens
  MISC_FEATURE: LIGHT CHAIN VL
  MISC_FEATURE: LIGHT CHAIN VL FAB1
SYVLTQPPSVSVAPGQTARITCGGNNLGSKSVHWYQQKPGQAPVLVVYDDSDRPSWIPERFSGSNSGNTATLTISRGEAGDEADYYCQVWDSSSDHVVFGGGTKLTVL

SEQ ID NO: 9 - DNA, 366 bp, Homo sapiens
  misc_feature: VARIABLE HEAVY CHAIN FAB1
cagatgcagttggttgaatctggtggcggcgtggtgcagcctggcagatctctgagactgtcttgtgccgcctccggcttcaccttcagaacctacggaatgcactgggtccgacaggcccctggcaaaggattggaatgggtcgccgtgatttggtacgacggctccaacaagcactacgccgactccgtgaagggcagattcaccatcaccagagacaactccaagaacaccctgaacctgcagatgaactccctgagagccgaggacaccgccgtgtactattgtgctagagcccctcagtgggaactcgtgcatgaggcctttgacatctggggccagggaacaatggtcaccgtctcctca

SEQ ID NO: 10 - DNA, 324 bp, Homo sapiens
  misc_feature: FAB1 VARIABLE LIGHT CHAIN
tcatatgttcttacacaaccaccgtcggtttcggttgctccaggacaaacagctcgaattacatgcggaggaaacaacctcggatcgaagtcggttcactggtatcaacaaaagccaggacaagctccagttctcgtggtgtacgatgattcagatcgaccatcatggatcccagagcgattctcaggatcaaactcgggaaatactgccacgctcacaatttcacgcggagaagcgggagatgaagctgattactattgccaagtgtgggactcgtcgtcagatcatgttgttttcggaggtggaacaaagctcacagtgctc

SEQ ID NO: 11 - protein, 11 aa, Homo sapiens
  MISC_FEATURE: LCDR1 FAB2
GGNNIGSKSVH

SEQ ID NO: 12 - protein, 108 aa, Homo sapiens
  MISC_FEATURE: LIGHT CHAIN FAB2
  MISC_FEATURE: LIGHT CHAIN VL FAB2
SYVLTQPPSVSVAPGQTARITCGGNNIGSKSVHWYQQKPGQAPVLVVYDDSDRPSWIPERFSGSNSGNTATLTISRGEAGDEADYYCQVWDSSSDHVVFGGGTKLTVL

SEQ ID NO: 13 - protein, 11 aa, Homo sapiens
  MISC_FEATURE: LCDR1 FAB3
GGNNVGSKSVH

SEQ ID NO: 14 - protein, 108 aa, Homo sapiens
  MISC_FEATURE: LIGHT CHAIN FAB3
  MISC_FEATURE: LIGHT CHAIN VL FAB3
SYVLTQPPSVSVAPGQTARITCGGNNVGSKSVHWYQQKPGQAPVLVVYDDSDRPSWIPERFSGSNSGNTATLTISRGEAGDEADYYCQVWDSSSDHVVFGGGTKLTVL

SEQ ID NO: 15 - protein, 17 aa, Homo sapiens
  MISC_FEATURE: HCDR2 FAB4
VIWYDGSNKHYAESVKG

SEQ ID NO: 16 - protein, 122 aa, Homo sapiens
  MISC_FEATURE: HEAVY CHAIN FAB4
  MISC_FEATURE: HEAVY CHAIN VH FAB4
QMQLVESGGGVVQPGRSLRLSCAASGFTFRTYGMHWVRQAPGKGLEWVAVIWYDGSNKHYAESVKGRFTITRDNSKNTLNLQMNSLRAEDTAVYYCARAPQWELVHEAFDIWGQGTMVTVSS

SEQ ID NO: 17 - protein, 17 aa, Homo sapiens
  MISC_FEATURE: HCDR2 FAB5
VIWYDGSNKHYADSVKA

SEQ ID NO: 18 - protein, 122 aa, Homo sapiens
  MISC_FEATURE: HEAVY CHAIN FAB5
  MISC_FEATURE: HEAVY CHAIN VH FAB5
QMQLVESGGGVVQPGRSLRLSCAASGFTFRTYGMHWVRQAPGKGLEWVAVIWYDGSNKHYADSVKARFTITRDNSKNTLNLQMNSLRAEDTAVYYCARAPQWELVHEAFDIWGQGTMVTVSS

SEQ ID NO: 19 - protein, 11 aa, Homo sapiens
  MISC_FEATURE: LCDR1 FAB6
GGQNLGSKSVH

SEQ ID NO: 20 - protein, 108 aa, Homo sapiens
  MISC_FEATURE: LIGHT CHAIN FAB6
  MISC_FEATURE: LIGHT CHAIN VL FAB6
SYVLTQPPSVSVAPGQTARITCGGQNLGSKSVHWYQQKPGQAPVLVVYDDSDRPSWIPERFSGSNSGNTATLTISRGEAGDEADYYCQVWDSSSDHVVFGGGTKLTVL

SEQ ID NO: 21 - protein, 11 aa, Homo sapiens
  MISC_FEATURE: LCDR1 FAB7
GGNQLGSKSVH

SEQ ID NO: 22 - protein, 108 aa, Homo sapiens
  MISC_FEATURE: LIGHT CHAIN FAB7
  MISC_FEATURE: LIGHT CHAIN VL FAB7
SYVLTQPPSVSVAPGQTARITCGGNQLGSKSVHWYQQKPGQAPVLVVYDDSDRPSWIPERFSGSNSGNTATLTISRGEAGDEADYYCQVWDSSSDHVVFGGGTKLTVL

SEQ ID NO: 23 - protein, 11 aa, Homo sapiens
  MISC_FEATURE: LCDR3 FAB8
QVWDTSSDHVV

SEQ ID NO: 24 - protein, 108 aa, Homo sapiens
  MISC_FEATURE: LIGHT CHAIN FAB8
  MISC_FEATURE: LIGHT CHAIN VL FAB8
SYVLTQPPSVSVAPGQTARITCGGNNLGSKSVHWYQQKPGQAPVLVVYDDSDRPSWIPERFSGSNSGNTATLTISRGEAGDEADYYCQVWDTSSDHVVFGGGTKLTVL

SEQ ID NO: 25 - protein, 11 aa, Homo sapiens
  MISC_FEATURE: LCDR3 FAB9
QVWDSTSDHVV

SEQ ID NO: 26 - protein, 108 aa, Homo sapiens
  MISC_FEATURE: LIGHT CHAIN FAB9
  MISC_FEATURE: LIGHT CHAIN VL FAB9
SYVLTQPPSVSVAPGQTARITCGGNNLGSKSVHWYQQKPGQAPVLVVYDDSDRPSWIPERFSGSNSGNTATLTISRGEAGDEADYYCQVWDSTSDHVVFGGGTKLTVL

SEQ ID NO: 27 - protein, 159 aa, homo sapiens
MFPFALLYVLSVSFRKIFILQLVGLVLTYDFTNCDFEKIKAAYLSTISKDLITYMSGTKSTEFNNTVSCSNRPHCLTEIQSLTFNPTAGCASLAKEMFAMKTKAALAIWCPGYSETQINATQAMKKRRKRKVTTNKCLEQVSQLQGLWRRFNRPLLKQQ

SEQ ID NO: 28 - protein, 227 aa, Homo Sapiens
QMQLVESGGGVVQPGRSLRLSCAASGFTFRTYGMHWVRQAPGKGLEWVAVIWYDGSNKHYADSVKGRFTITRDNSKNTLNLQMNSLRAEDTAVYYCARAPQWELVHEAFDIWGQGTMVTVSSASTKGPSVFPLAPSSKSTSGGTAALGCLVKDYFPEPVTVSWNSGALTSGVHTFPAVLQSSGLYSLSSVVTVPSSSLGTQTYICNVNHKPSNTKVDKRVEPKSCDK

SEQ ID NO: 29 - protein, 214 aa, Homo Sapiens
SYVLTQPPSVSVAPGQTARITCGGNNLGSKSVHWYQQKPGQAPVLVVYDDSDRPSWIPERFSGSNSGNTATLTISRGEAGDEADYYCQVWDSSSDHVVFGGGTKLTVLGQPKAAPSVTLFPPSSEELQANKATLVCLISDFYPGAVTVAWKADSSPVKAGVETTTPSKQSNNKYAASSYLSLTPEQWKSHRSYSCQVTHEGSTVEKTVAPTECS

SEQ ID NO: 30 - DNA, 681 bp, Homo sapiens
cagatgcagttggttgaatctggtggcggcgtggtgcagcctggcagatctctgagactgtcttgtgccgcctccggcttcaccttcagaacctacggaatgcactgggtccgacaggcccctggcaaaggattggaatgggtcgccgtgatttggtacgacggctccaacaagcactacgccgactccgtgaagggcagattcaccatcaccagagacaactccaagaacaccctgaacctgcagatgaactccctgagagccgaggacaccgccgtgtactattgtgctagagcccctcagtgggaactcgtgcatgaggcctttgacatctggggccagggaacaatggtcaccgtctcctcagcctccaccaagggcccatcggtcttccccctggcaccctcctccaagagcacctctgggggcacagcggccctgggctgcctggtcaaggactacttccccgaaccggtgacggtgtcgtggaactcaggcgccctgaccagcggcgtgcacaccttcccggctgtcctacagtcctcaggactctactccctcagcagcgtggtgacagtgccctccagcagcttgggcacccagacctacatctgcaacgtgaatcacaagcccagcaacaccaaggtggacaagagagttgagcccaaatcttgtgacaaa

SEQ ID NO: 31 - DNA, 642 bp, Homo sapiens
tcatatgttcttacacaaccaccgtcggtttcggttgctccaggacaaacagctcgaattacatgcggaggaaacaacctcggatcgaagtcggttcactggtatcaacaaaagccaggacaagctccagttctcgtggtgtacgatgattcagatcgaccatcatggatcccagagcgattctcaggatcaaactcgggaaatactgccacgctcacaatttcacgcggagaagcgggagatgaagctgattactattgccaagtgtgggactcgtcgtcagatcatgttgttttcggaggtggaacaaagctcacagtgctcggtcagcccaaggctgccccctcggtcactctgttcccgccctcctctgaggagcttcaagccaacaaggccacactggtgtgtctcataagtgacttctacccgggagccgtgacagtggcctggaaggcagatagcagccccgtcaaggcgggagtggagaccaccacaccctccaaacaaagcaacaacaagtacgcggccagcagctatctgagcctgacgcctgagcagtggaagtcccacagaagctacagctgccaggtcacgcatgaagggagcaccgtggagaagacagtggcccctacagaatgttca